European Patent Specification EP 3 971 169 B1, published May 27, 2026. Title: REAGENTS AND METHODS FOR BIOORTHOGONAL LABELING OF BIOMOLECULES IN LIVING CELLS. Applicant: OREGON STATE UNIVERSITY. The sequence listing filed with the application follows.

SEQUENCE LISTING (7 sequences)

SEQ ID NO: 1 - DNA, 26 bp, Artificial Sequence
  Synthetic
cgcgcgccatggacgaatttgaaatg

SEQ ID NO: 2 - DNA, 37 bp, Artificial Sequence
  Synthetic
gactcagtctaggtacccgtttgaaactgcagttata

SEQ ID NO: 3 - DNA, 25 bp, Artificial Sequence
  Synthetic
cttcctggaaatcaagagccccatc

SEQ ID NO: 4 - DNA, 20 bp, Artificial Sequence
  Synthetic
gttccaggtcgccgtgcatg

SEQ ID NO: 5 - DNA, 18 bp, Artificial Sequence
  Synthetic
tgcacggcgacctggaac

SEQ ID NO: 6 - DNA, 22 bp, Artificial Sequence
  Synthetic
ggggctcttgatttccaggaag

SEQ ID NO: 7 - DNA, 22 bp, Artificial Sequence
  Synthetic
catgtaggcctgataagcgtag